European Patent Specification EP 4 058 598 B1, published April 23, 2025. Title: GENERATING CAPTURE PROBES FOR SPATIAL ANALYSIS. Applicant: 10x Genomics, Inc. The sequence listing filed with the application follows.

SEQUENCE LISTING (34 sequences)

SEQ ID NO: 1 - protein, 16 aa, Artificial
  Synthetic polypeptide
RADARADARADARADA

SEQ ID NO: 2 - protein, 16 aa, Artificial
  Synthetic EAK16 polypeptide
AEAEAKAKAEAEAKAK

SEQ ID NO: 3 - protein, 12 aa, Artificial
  Synthetic KLD12 polypeptide
KLDLKLDLKLDL

SEQ ID NO: 4 - DNA, 18 bp, Artificial
  18s cDNA Probe 1
gaggaattcccagtaagt

SEQ ID NO: 5 - DNA, 18 bp, Artificial
  18S cDNA Probe 2
gagattgagcaataacag

SEQ ID NO: 6 - DNA, 18 bp, Artificial
  18s cDNA Probe 3
gtagttccgaccataaac

SEQ ID NO: 7 - DNA, 18 bp, Artificial
  18s cDNA Probe 4
ggtgactctagataacct

SEQ ID NO: 8 - RNA, 35 nt, Artificial
  Analyte poly(A) tail from biological sample
  misc_feature (12)..(35): n is a, c, g, or u
aaaaaaaaaaannnnnnnnnnnnnnnnnnnnnnnn

SEQ ID NO: 9 - DNA, 8 bp, Artificial
  Acceptor Oligonucleotide Ligation Handle
gcggcccg

SEQ ID NO: 10 - DNA, 18 bp, Artificial
  Splint Oligonucleotide
aaaaaaaaaacgggccgc

SEQ ID NO: 11 - DNA, 27 bp, Artificial
  Capture domain poly(T) sequence
ttttttttttttttttttttttttttt

SEQ ID NO: 12 - DNA, 7 bp, Artificial
  Acceptor Oligonucleotide Ligation Handle 2
cgctacg

SEQ ID NO: 13 - DNA, 14 bp, Artificial
  Universal Splint Oligonucleotide
tcgactacgtagcg

SEQ ID NO: 14 - DNA, 7 bp, Artificial
  Acceptor Oligonucleotide 3
cgctacg

SEQ ID NO: 15 - DNA, 37 bp, Artificial
  T30VN
tagtcgatttttttttttttttttttttttttttttt

SEQ ID NO: 16 - DNA, 13 bp, Artificial
  N6 Random
  misc_feature (8)..(13): n is a, c, g, or t
tagtcgannnnnn

SEQ ID NO: 17 - DNA, 16 bp, Artificial
  N9 Random
  misc_feature (8)..(16): n is a, c, g, or t
tagtcgannnnnnnnn

SEQ ID NO: 18 - DNA, 19 bp, Artificial
  N12 Random
  misc_feature (8)..(19): n is a, c, g, or t
tagtcgannnnnnnnnnnn

SEQ ID NO: 19 - DNA, 28 bp, Artificial
  Capture Sequence with Ligation Handle
tagtcgattgctaggaccggccttaagc

SEQ ID NO: 20 - DNA, 21 bp, Artificial
  Capture Sequence Domain of Capture Sequence
ttgctaggaccggccttaagc

SEQ ID NO: 21 - DNA, 22 bp, Artificial
  Splint Oligonucleotide V2-1
gctagtaaggtgcgcaatcctc

SEQ ID NO: 22 - DNA, 22 bp, Artificial
  Splint Oligonucleotide V2-2
gcaccttggaccgctaaagttg

SEQ ID NO: 23 - DNA, 22 bp, Artificial
  Splint Oligonucleotide V2-3
gctagtcgagccgacaattgtc

SEQ ID NO: 24 - DNA, 22 bp, Artificial
  Splint Oligonucleotide V2-4
gcctgacgaaccggttttgcaa

SEQ ID NO: 25 - DNA, 55 bp, Artificial
  Donor Oligonucleotide UMI-V2-1
  misc_feature (12)..(23): n is a, c, g, or t
  misc_feature (55)..(55): n is a, c, g, or t
accttactagcnnnnnnnnnnnnttttttttttttttttttttttttttttttvn

SEQ ID NO: 26 - DNA, 55 bp, Artificial
  Donor Oligonucleotide UMI-V2-2
  misc_feature (12)..(23): n is a, c, g, or t
  misc_feature (55)..(55): n is a, c, g, or t
gtccaaggtgcnnnnnnnnnnnnttttttttttttttttttttttttttttttvn

SEQ ID NO: 27 - DNA, 55 bp, Artificial
  Donor Oligonucleotide UMI-V2-3
  misc_feature (12)..(23): n is a, c, g, or t
  misc_feature (55)..(55): n is a, c, g, or t
gctcgactagcnnnnnnnnnnnnttttttttttttttttttttttttttttttvn

SEQ ID NO: 28 - DNA, 55 bp, Artificial
  Donor Oligonucleotide UMI-V2-4
  misc_feature (12)..(23): n is a, c, g, or t
  misc_feature (55)..(55): n is a, c, g, or t
gttcgtcaggcnnnnnnnnnnnnttttttttttttttttttttttttttttttvn

SEQ ID NO: 29 - DNA, 55 bp, Artificial; identical to SEQ ID NO: 25
  Donor Oligonucleotide UMI-Cy3
  misc_feature (12)..(23): n is a, c, g, or t
  misc_feature (55)..(55): n is a, c, g, or t

SEQ ID NO: 30 - DNA, 11 bp, Artificial
  Acceptor Oligonucleotide Ligation Handle V2-1
gaggattgcgc

SEQ ID NO: 31 - DNA, 11 bp, Artificial
  Acceptor Oligonucleotide Ligation Handle V2-2
caactttagcg

SEQ ID NO: 32 - DNA, 11 bp, Artificial
  Acceptor Oligonucleotide Ligation Handle V2-3
gacaattgtcg

SEQ ID NO: 33 - DNA, 9 bp, Artificial
  Acceptor Oligonucleotide Ligation Handle V2-4
gcaaaaccg

SEQ ID NO: 34 - DNA, 22 bp, Artificial
  Blocking Probe
agatcggaagagcgtcgtgtag